European Patent Specification EP 3 325 029 B1, published May 24, 2023. Title: SOY-DERIVED BIOACTIVE PEPTIDES FOR USE IN COMPOSITIONS AND METHODS FOR WOUND HEALING, TISSUE ENGINEERING, AND REGENERATIVE MEDICINE. Applicant: Temple University Lelkes, Peter Har-el, Yah-el Marcinkiewicz, Cezary Lazarovici, Philip Baharlou, Sogol Gerstenhaber, Jonathon. The sequence listing filed with the application follows.

SEQUENCE LISTING (64 sequences)

SEQ ID NO: 1 - protein, 8 aa, Artificial Sequence
  LDV
EILDVPST

SEQ ID NO: 2 - protein, 8 aa, Artificial Sequence
  CS-1
RDLDVFLS

SEQ ID NO: 3 - protein, 559 aa, Artificial Sequence
  beta-conglycinin subunit alpha, partial
VEEEEECEEGQIPRPRPQHPERERQQHGEKEEDEGEQPRPFPFPRPRQPHQEEEHEQKEEHEWHRKEEKEGGKGSEEEQDEREHPRPHQPHQKEEEKHEWQHKQEKHQGKESEEEEEDQDEDEEQDKESQESEGSESQREPRRHKNKNPFHFNSKRFQTLFKNQYGHVRVLQRFNKRSQQLQNLRDYRILEFNSKPNTLLLPHHADADYLIVILNGTALLTLVNNDDRDSYNLQSGDALRVPAGTTYYVVNPDNDENLRMITLAIPVNKPGRFESFFLSSTQAQQSYLQGFSKNILEASYDTKFEEINKVLFGREEGQQQGEERLQESVIVEISKKQIRELSKHAKSSSRKTISSEDKPFNLRSRDPIYSNKLGKLFEITPEKNPQLRDLDVFLSVVDMNEGALFLPHFNSKAIVVLVINEGEANIELVGIKEQQQRQQQEFQPLEVRKYRAELSEQDIFVIPAGYPVVVNATSDLNFFAFGINAENNQRNFLAGSKDNVISQIPSQVQELAFPGSAKDIENLIKSQSESYFVDAQPQQKEEGNKGRKGPLSSILRAFY

SEQ ID NO: 4 - protein, 114 aa, Artificial Sequence
  BCF9-4
SQQLQNLRDSYNLQSGDALRVPAGTTYYVVNPDNDENLRMITLAIPVNKPGRNILEASYDTKVLFGREEGQQQGEERTISSEDKPFNLRDELPQLVTLPHPSLHGPEILDVPST

SEQ ID NO: 5 - protein, 37 aa, Artificial Sequence
  BCF9-4
LQSGDALRNILEASYDTKFEEINKKTISSEDKPFNLR

SEQ ID NO: 6 - protein, 25 aa, Artificial Sequence
  CS-1
DELPQLVTLPHPSLHGPEILDVPST

SEQ ID NO: 7 - protein, 22 aa, Artificial Sequence
  BCF5-4A
QHGNTGGLYYGTDTADTGTGPR

SEQ ID NO: 8 - protein, 9 aa, Artificial Sequence
  BCF5-4A
VGATVMINI

SEQ ID NO: 9 - protein, 14 aa, Artificial Sequence
  BCF5-4A
YYGTNTADTGTGPR

SEQ ID NO: 10 - protein, 10 aa, Artificial Sequence
  BCF5-4A
HAAWTYVATR

SEQ ID NO: 11 - protein, 13 aa, Artificial Sequence
  BCF5-4B
QGETVVPGGTGGK

SEQ ID NO: 12 - protein, 10 aa, Artificial Sequence
  BCF5-4B
KVDEYGNVEK

SEQ ID NO: 13 - protein, 14 aa, Artificial Sequence
  BCF5-4B
HHGTTGVYGIDTDR

SEQ ID NO: 14 - protein, 20 aa, Artificial Sequence
  BCF5-4B
QTDEYGNPVHAASVTYVATR

SEQ ID NO: 15 - protein, 22 aa, Artificial Sequence
  BCF5-4B
QHGNIGGPYYGTNTADTGTGPR

SEQ ID NO: 16 - protein, 7 aa, Artificial Sequence
  BCF5-4B
QCAHVCR

SEQ ID NO: 17 - protein, 7 aa, Artificial Sequence
  BCF5-4B
CFCSRPC

SEQ ID NO: 18 - protein, 10 aa, Artificial Sequence
  BCF5-4B
SDGFIGGQCR

SEQ ID NO: 19 - protein, 15 aa, Artificial Sequence
  BCF5-4B
QIVTVEGGLSVISPK

SEQ ID NO: 20 - protein, 16 aa, Artificial Sequence
  BCF5-4B
QQHDAIGVYPGIDIGR

SEQ ID NO: 21 - protein, 22 aa, Artificial Sequence
  BCF5-4B
QHGNTGGLYYGTDTADTGTGPR

SEQ ID NO: 22 - protein, 8 aa, Artificial Sequence
  BCF5-4C
ELMNLAIR

SEQ ID NO: 23 - protein, 13 aa, Artificial Sequence
  BCF5-4C
LGPMIGCDLSSDD

SEQ ID NO: 24 - protein, 15 aa, Artificial Sequence
  BCF5-4C
CRLGPMIGCDLSSDD

SEQ ID NO: 25 - protein, 7 aa, Artificial Sequence
  BCF5-4D
QCAHVCR

SEQ ID NO: 26 - protein, 7 aa, Artificial Sequence
  BCF5-4D
CFCSRPC

SEQ ID NO: 27 - protein, 10 aa, Artificial Sequence
  BCF5-4D
SDGFIGGQCR

SEQ ID NO: 28 - protein, 12 aa, Artificial Sequence
  BCF5-4D
CLFDRQCAHVCR

SEQ ID NO: 29 - protein, 12 aa, Artificial Sequence
  BCF5-4D
SMPPQCSCEDIR

SEQ ID NO: 30 - protein, 13 aa, Artificial Sequence
  BCF5-4D
CLDTNDFCYKPCK

SEQ ID NO: 31 - protein, 8 aa, Artificial Sequence
  BCF5-4D
CGVNIPYK

SEQ ID NO: 32 - protein, 15 aa, Artificial Sequence
  BCF5-4D
DEYSKPCCDLCMCTR

SEQ ID NO: 33 - protein, 13 aa, Artificial Sequence
  BCF5-5
LGPMIGCDLSSDD

SEQ ID NO: 34 - protein, 12 aa, Artificial Sequence
  BCF5-5
IMDNQSEQLEGK

SEQ ID NO: 35 - protein, 13 aa, Artificial Sequence
  BCF5-5
KQMERELMNLAIR

SEQ ID NO: 36 - protein, 15 aa, Artificial Sequence
  BCF5-5
CRLGPMIGCDLSSDD

SEQ ID NO: 37 - protein, 16 aa, Artificial Sequence
  BCF5-5
CCSEMSELKSPICQCK

SEQ ID NO: 38 - protein, 15 aa, Artificial Sequence
  BCF5-5
QIVTVEGGLSVISPK

SEQ ID NO: 39 - protein, 8 aa, Artificial Sequence
  BCF9-4
SQQLQNLR

SEQ ID NO: 40 - protein, 10 aa, Artificial Sequence
  BCF9-4
NILEASYDTK

SEQ ID NO: 41 - protein, 12 aa, Artificial Sequence
  BCF9-4
DSYNLQSGDALR

SEQ ID NO: 42 - protein, 12 aa, Artificial Sequence
  BCF9-4
TISSEDKPFNLR

SEQ ID NO: 43 - protein, 13 aa, Artificial Sequence
  BCF9-4
MITLAIPVNKPGR

SEQ ID NO: 44 - protein, 13 aa, Artificial Sequence
  BCF9-4
KTISSEDKPFNLR

SEQ ID NO: 45 - protein, 15 aa, Artificial Sequence
  BCF9-4
VLFGREEGQQQGEER

SEQ ID NO: 46 - protein, 16 aa, Artificial Sequence
  BCF9-4
NILEASYDTKFEEINK

SEQ ID NO: 47 - protein, 19 aa, Artificial Sequence
  BCF9-4
VPAGTTYYVVNPDNDENLR

SEQ ID NO: 48 - protein, 8 aa, Artificial Sequence
  BCF9-4
LQSGDALR

SEQ ID NO: 49 - protein, 13 aa, Artificial Sequence
  BCF9-4
LITLAIPVNKPGR

SEQ ID NO: 50 - protein, 19 aa, Artificial Sequence
  BCF9-4
VPSGTTYYVVNPDNNENLR

SEQ ID NO: 51 - protein, 13 aa, Artificial Sequence
  BCF9-4
ISTLNSLTLPALR

SEQ ID NO: 52 - protein, 19 aa, Artificial Sequence
  BCF9-4
AIPSEVLSNSYNLGQSQVR

SEQ ID NO: 53 - protein, 17 aa, Artificial Sequence
  BCF9-4
FNECQLNNLNALEPDHR

SEQ ID NO: 54 - protein, 8 aa, Artificial Sequence
  BCF9-5
LQSGDALR

SEQ ID NO: 55 - protein, 8 aa, Artificial Sequence
  BCF9-5
SPQLQNLR

SEQ ID NO: 56 - protein, 10 aa, Artificial Sequence
  BCF9-5
NILEASYDTK

SEQ ID NO: 57 - protein, 13 aa, Artificial Sequence
  BCF9-5
LITLAIPVNKPGR

SEQ ID NO: 58 - protein, 12 aa, Artificial Sequence
  BCF9-5
TISSEDKPFNLR

SEQ ID NO: 59 - protein, 15 aa, Artificial Sequence
  BCF9-5
LQESVIVEISKEQIR

SEQ ID NO: 60 - protein, 15 aa, Artificial Sequence
  BCF9-5
VLFSREEGQQQGEQR

SEQ ID NO: 61 - protein, 19 aa, Artificial Sequence
  BCF9-5
VPSGTTYYVVNPDNNENLR

SEQ ID NO: 62 - protein, 8 aa, Artificial Sequence
  BCF9-5
SQQLQNLR

SEQ ID NO: 63 - protein, 13 aa, Artificial Sequence
  BCF9-5
MITLAIPVNKPGR

SEQ ID NO: 64 - protein, 19 aa, Artificial Sequence
  BCF9-5
VPAGTTYYVVNPDNDENLR